European Patent Specification EP 3 010 933 B1, published May 15, 2024. Title: ANTICORPS MONOCATÉNAIRE À CHAÎNE LOURDE DE CAMÉLIDÉ DIRIGÉ CONTRE LA CHROMATINE ET UTILISATIONS. Applicant: INSTITUT NATIONAL DE LA RECHERCHE AGRONOMIQUE UNIVERSITE PAUL SABATIER TOULOUSE III. The sequence listing filed with the application follows.

SEQUENCE LISTING (13 sequences)

SEQ ID NO: 1 - protein, 125 aa, Lama glama
MAQVQLQASGGGLVQAGDSLRLSCAAAGRSFSSYAMGWFRQAPGKEREFVAAISRSRGVTYADSVKGRFTISKDNVKNMAYLQMNSLKPEDTGVYYCAATSSGSTRQLSTGRSNYWGQGTQVTVS

SEQ ID NO: 2 - protein, 123 aa, Lama glama
MAQVQLQASGGGLVQAGGSLRLSCAASGRTVATLGWFRQAPGKEREFVAGITWTAGRTYYADSVKGRFTISRDNKRTTYLQMNSLKPEDTGVYYCAATSSGSTRLLSTGRDNYWGQGTLVTVS

SEQ ID NO: 3 - protein, 122 aa, Lama glama
MAQVQLQASGGGLVQAGESLTLSCDASGRTFSIGAMGWFRQAPGKEREFLAAINWNGGYTSYADVASGRFTISRNAKNTVYLQMNSLQPEDTAVYYCAAKYGGSARSRTYDYWGQGTQVTVS

SEQ ID NO: 4 - protein, 121 aa, Lama glama
MAQVQLQASGGGLVQAGGSLRLSCAVSGGTLSSYTMGWFRQAPGKEREFVSALSRVGGKSDYADSVKGRFTISRNAKNTVYLQMNSLKPEDTAVYYCAAGGYSRRWSAYNYWGQGTQVTVS

SEQ ID NO: 5 - protein, 127 aa, Lama glama
MAEVQLQASGGGLVQPGNSLRLSCVGSGVSLSAYNMGWFRQAPGKEREFVADINVSGGTAYYADSVKGRFTISRDNVKNTLYLQMNSLKLDDAAVYYCAAAPAWRPFTYDSRDDYPYWGQGTQVTVS

SEQ ID NO: 6 - protein, 10 aa, Artificial sequence
  Phospho-peptide  H2AX synthétique
  MOD_RES (7)..(7): PHOSPHORYLATION
KKATQASQEY

SEQ ID NO: 7 - DNA, 23 bp, Artificial sequence
  Amorce PCR CALL01
gtcctggctgctcttctacaagg

SEQ ID NO: 8 - DNA, 23 bp, Artificial sequence
  Amorce PCR CALL02
ggtacgtgctgttgaactgttcc

SEQ ID NO: 9 - DNA, 23 bp, Artificial sequence
  Amorce PCR For
acggtacctcgggccgcggcaag

SEQ ID NO: 10 - DNA, 28 bp, Artificial sequence
  Amorce PCR Rev
cggatccctattagtactcctgggaggc

SEQ ID NO: 11 - protein, 30 aa, Artificial sequence
  Tag 2xStrep
WSHPQFEKGGGSGGGSGGGGSAWSHPQFEK

SEQ ID NO: 12 - DNA, 32 bp, Artificial sequence
  Amorce PCR N1VHH-F
atactcgagccaccatggcccaggtgcagctg

SEQ ID NO: 13 - DNA, 31 bp, Artificial sequence
  Amorce PCR N1VHH-R
aatggatccgcgtagtccggaacgtcgtacg